European Patent Application EP 4 763 859 A1, published June 24, 2026. Title: 一种具有抗衰功效的重组人源弹性蛋白及其组合物的应用. Applicant: 杭州恩和生物科技有限公司. The sequence listing filed with the application follows.

SEQUENCE LISTING (41 sequences)

SEQ ID NO: 1 - protein, 100 aa, synthetic construct
VTFPGALVPGGVADAAAAYKAAKAGAGLGGVPGVGGLGVSAGAVVPQPGAGVKPGKVPGVGLPGVYPGGVLPGARFPGVGVLPGVPTGAGVKPKAPGVGG

SEQ ID NO: 2 - protein, 89 aa, synthetic construct
MRFPSIFTAVLFAASSALAAPVNTTTEDETAQIPAEAVIGYLDLEGDFDVAVLPFSNSTNNGLLFINTTIASIAAKEEGVSLDKREAEA

SEQ ID NO: 3 - DNA, 597 bp, synthetic construct
  source 1..597: mol_type = other DNA
atgagattcccatctattttcactgctgttttgttcgctgcttcttctgctttggctgctccagttaacactactactgaggacgagactgctcaaattccagctgaggctgttattggttacttggacttggagggtgacttcgacgttgctgttttgccattctctaactctactaacaacggtttgttgttcattaacactactattgcttctattgctgctaaggaggagggtgtttctttggacaagagagaggctgaggctgttacattcccaggtgccctggttcctggcggagtcgctgatgctgctgcagcctataaagcagctaaagccggagccggtttaggtggtgtgccaggggtgggaggattaggtgtttcggcaggcgctgtcgttcctcaacccggagccggggtgaagcccggaaaagttcctggagtggggcttcctggagtttaccctggcggtgttttgcctggagccaggtttccgggtgttggtgttttgcccggagttccgactggcgccggtgtcaaacctaaagctccaggtgtgggtggtggcagttcacatcatcatcatcatcattag

SEQ ID NO: 4 - DNA, 939 bp, synthetic construct
  source 1..939: mol_type = other DNA
gatctaacatccaaagacgaaaggttgaatgaaacctttttgccatccgacatccacaggtccattctcacacataagtgccaaacgcaacaggaggggatacactagcagcagaccgttgcaaacgcaggacctccactcctcttctcctcaacacccacttttgccatcgaaaaaccagcccagttattgggcttgattggagctcgctcattccaattccttctattaggctactaacaccatgactttattagcctgtctatcctggcccccctggcgaggttcatgtttgtttatttccgaatgcaacaagctccgcattacacccgaacatcactccagatgagggctttctgagtgtggggtcaaatagtttcatgttccccaaatggcccaaaactgacagtttaaacgctgtcttggaacctaatatgacaaaagcgtgatctcatccaagatgaactaagtttggttcgttgaaatgctaacggccagttggtcaaaaagaaacttccaaaagtcggcataccgtttgtcttgtttggtattgattgacgaatgctcaaaaataatctcattaatgcttagcgcagtctctctatcgcttctgaaccccggtgcacctgtgccgaaacgcaaatggggaaacacccgctttttggatgattatgcattgtctccacattgtatgcttccaagattctggtgggaatactgctgatagcctaacgttcatgatcaaaatttaactgttctaacccctacttgacagcaatatataaacagaaggaagctgccctgtcttaaacctttttttttatcatcattattagcttactttcataattgcgactggttccaattgacaagcttttgattttaacgacttttaacgacaacttgagaagatcaaaaaacaactaattattcgaaacg

SEQ ID NO: 5 - DNA, 350 bp, synthetic construct
  source 1..350: mol_type = other DNA
tcaagaggatgtcagaatgccatttgcctgagagatgcaggcttcatttttgatacttttttatttgtaacctatatagtataggattttttttgtcattttgtttcttctcgtacgagcttgctcctgatcagcctatctcgcagctgatgaatatcttgtggtaggggtttgggaaaatcattcgagtttgatgtttttcttggtatttcccactcctcttcagagtacagaagattaagtgacacgttcgtttgtgcaagcttcaacgatgccaaaagggtataataagcgtcatttgcagcattgtgaagaaaactatgtggcaagccaagcctgcgaagaatgta

SEQ ID NO: 6 - DNA, 1426 bp, synthetic construct
  source 1..1426: mol_type = other DNA
agcttgcctcgtccccgccgggtcacccggccagcgacatggaggcccagaataccctccttgacagtcttgacgtgcgcagctcaggggcatgatgtgactgtcgcccgtacatttagcccatacatccccatgtataatcatttgcatccatacattttgatggccgcacggcgcgaagcaaaaattacggctcctcgctgcagacctgcgagcagggaaacgctcccctcacagacgcgttgaattgtccccacgccgcgcccctgtagagaaatataaaaggttaggatttgccactgaggttcttctttcatatacttccttttaaaatcttgctaggatacagttctcacatcacatccgaacataaacaaaaatgggtaaggaaaagactcacgtttccagaccaagattgaactctaacatggacgctgacttgtacggttacaagtgggctagagacaacgttggtcaatctggtgctactatttacagattgtacggtaagccagacgctccagagttgttcttgaagcacggtaagggttctgttgctaacgacgttactgacgagatggttagattgaactggttgactgagttcatgccattgccaactattaagcacttcattagaactccagacgacgcttggttgttgactactgctattccaggtaagactgctttccaagttttggaggagtacccagactctggtgagaacattgttgacgctttggctgttttcttgagaagattgcactctattccagtttgtaactgtccattcaactctgacagagttttcagattggctcaagctcaatccagaatgaacaacggtttggttgacgcttctgacttcgacgacgagagaaacggttggccagttgagcaagtttggaaggagatgcacaagttgttgccattctctccagactctgttgttactcacggtgacttctctttggacaacttgattttcgacgagggtaagttgattggttgtattgacgttggtagagttggtattgctgacagataccaagacttggctattttgtggaactgtttgggtgagttctctccatctttgcaaaagagattgttccaaaagtacggtattgacaacccagacatgaacaagttgcaattccacttgatgttggacgagttcttctaaagtaactgacaataaaaagattcttgttttcaagaacttgtcatttgtatagtttttttatattgtagttgttctattttaatcaaatgttagcgtgatttatattttttttcgcctcgacatcatctgcccagatgcgaagttaagtgcgcagaaagtaatatcatgcgtcaatcgtatgtgaatgctggtcgctatactgctgtcgattcgatactaacgccgccatccagtgtc

SEQ ID NO: 7 - DNA, 589 bp, synthetic construct
  source 1..589: mol_type = other DNA
ttgagatcctttttttctgcgcgtaatctgctgcttgcaaacaaaaaaaccaccgctaccagcggtggtttgtttgccggatcaagagctaccaactctttttccgaaggtaactggcttcagcagagcgcagataccaaatactgttcttctagtgtagccgtagttaggccaccacttcaagaactctgtagcaccgcctacatacctcgctctgctaatcctgttaccagtggctgctgccagtggcgataagtcgtgtcttaccgggttggactcaagacgatagttaccggataaggcgcagcggtcgggctgaacggggggttcgtgcacacagcccagcttggagcgaacgacctacaccgaactgagatacctacagcgtgagctatgagaaagcgccacgcttcccgaagggagaaaggcggacaggtatccggtaagcggcagggtcggaacaggagagcgcacgagggagcttccagggggaaacgcctggtatctttatagtcctgtcgggtttcgtcacctctgacttgagcgtcgatttttgtgatgctcgtcaggggggcggagcctatggaaa

SEQ ID NO: 8 - DNA, 1136 bp, synthetic construct
  source 1..1136: mol_type = other DNA
cgcggaacccctatttgtttatttttctaaatacattcaaatatgtatccgctcatgagacaataaccctgataaatgcttcaataatattgaaaaaggaagagtatgagtattcaacatttccgtgtcgcccttattcccttttttgcggcattttgccttcctgtttttgctcacccagaaacgctggtgaaagtaaaagatgctgaagatcagttgggtgcacgagtgggttacatcgaactggatctcaacagcggtaagatccttgagagttttcgccccgaagaacgttttccaatgatgagcacttttaaagttctgctatgtggcgcggtattatcccgtattgacgccgggcaagagcaactcggtcgccgcatacactattctcagaatgacttggttgagtactcaccagtcacagaaaagcatcttacggatggcatgacagtaagagaattatgcagtgctgccataaccatgagtgataacactgcggccaacttacttctgacaacgatcggaggaccgaaggagctaaccgcttttttgcacaacatgggggatcatgtaactcgccttgatcgttgggaaccggagctgaatgaagccataccaaacgacgagcgtgacaccacgatgcctgtagcaatggcaacaacgttgcgcaaactattaactggcgaactacttactctagcttcccggcaacaattaatagactggatggaggcggataaagtggccggcccacttctgcgctcggcccttccggccggctggtttattgctgataaatctggagccggtgagcgtggatctcgcggtatcattgcagcactggggccagatggtaagccctcccgtatcgtagttatctacacgacggggagtcaggcaactatggatgaacgaaatagacagatcgctgagataggtgcctcactgattaagcattggtaactgtcagaccaagtttactcatatatactttagattgatttaaatcttcatttttaattaaaaaggatctaggtgaagatcctttttgataatctcatgaccaaaatcccttaacgtgagttttcgttccactgagcgtcagaccccgtagaaaagatcaaaggatcttc

SEQ ID NO: 9 - DNA, 3252 bp, synthetic construct
  source 1..3252: mol_type = other DNA
gtcgagaattgagcttgcctcgtccccgccgggtcacccggccagcgacatggaggcccagaataccctccttgacagtcttgacgtgcgcagctcaggggcatgatgtgactgtcgcccgtacatttagcccatacatccccatgtataatcatttgcatccatacattttgatggccgcacggcgcgaagcaaaaattacggctcctcgctgcagacctgcgagcagggaaacgctcccctcacagacgcgttgaattgtccccacgccgcgcccctgtagagaaatataaaaggttaggatttgccactgaggttcttctttcatatacttccttttaaaatcttgctaggatacagttctcacatcacatccgaacataaacaaaaatgggtaaggaaaagactcacgtttccagaccaagattgaactctaacatggacgctgacttgtacggttacaagtgggctagagacaacgttggtcaatctggtgctactatttacagattgtacggtaagccagacgctccagagttgttcttgaagcacggtaagggttctgttgctaacgacgttactgacgagatggttagattgaactggttgactgagttcatgccattgccaactattaagcacttcattagaactccagacgacgcttggttgttgactactgctattccaggtaagactgctttccaagttttggaggagtacccagactctggtgagaacattgttgacgctttggctgttttcttgagaagattgcactctattccagtttgtaactgtccattcaactctgacagagttttcagattggctcaagctcaatccagaatgaacaacggtttggttgacgcttctgacttcgacgacgagagaaacggttggccagttgagcaagtttggaaggagatgcacaagttgttgccattctctccagactctgttgttactcacggtgacttctctttggacaacttgattttcgacgagggtaagttgattggttgtattgacgttggtagagttggtattgctgacagataccaagacttggctattttgtggaactgtttgggtgagttctctccatctttgcaaaagagattgttccaaaagtacggtattgacaacccagacatgaacaagttgcaattccacttgatgttggacgagttcttctaaagtaactgacaataaaaagattcttgttttcaagaacttgtcatttgtatagtttttttatattgtagttgttctattttaatcaaatgttagcgtgatttatattttttttcgcctcgacatcatctgcccagatgcgaagttaagtgcgcagaaagtaatatcatgcgtcaatcgtatgtgaatgctggtcgctatactgctgtcgattcgatactaacgccgccatccagtgtcggatctgtgagcaaaaggccagcaaaaggccaggaaccgtaaaaaggccgcgttgctggcgtttttccataggctccgcccccctgacgagcatcacaaaaatcgacgctcaagtcagaggtgacgaaacccgacaggactataaagataccaggcgtttccccctggaagctccctcgtgcgctctcctgttccgaccctgccgcttaccggatacctgtccgcctttctcccttcgggaagcgtggcgctttctcatagctcacgctgtaggtatctcagttcggtgtaggtcgttcgctccaagctgggctgtgtgcacgaaccccccgttcagcccgaccgctgcgccttatccggtaactatcgtcttgagtccaacccggtaagacacgacttatcgccactggcagcagccactggtaacaggattagcagagcgaggtatgtaggcggtgctacagagttcttgaagtggtggcctaactacggctacactagaagaacagtatttggtatctgcgctctgctgaagccagttaccttcggaaaaagagttggtagctcttgatccggcaaacaaaccaccgctggtagcggtggtttttttgtttgcaagcagcagattacgcgcagaaaaaaaggatctcaagaagatcctttgatcttttctacggggtctgacgctcagtggaacgaaaactcacgttaagggattttggtcatgagattatcaaaaaggatcttcacctagatcctttttaattaaaaatgaagatttaaatcaatctaaagtatatatgagtaaacttggtctgacagttaccaatgcttaatcagtgaggcacctatctcagcgatctgtctatttcgttcatccatagttgcctgactccccgtcgtgtagataactacgatacgggagggcttaccatctggccccagtgctgcaatgataccgcgagatccacgctcaccggctccagatttatcagcaataaaccagccggccggaagggccgagcgcagaagtgggccggccactttatccgcctccatccagtctattaattgttgccgggaagctagagtaagtagttcgccagttaatagtttgcgcaacgttgttgccattgctacaggcatcgtggtgtcacgctcgtcgtttggtatggcttcattcagctccggttcccaacgatcaaggcgagttacatgatcccccatgttgtgcaaaaaagcggttagctccttcggtcctccgatcgttgtcagaagtaagttggccgcagtgttatcactcatggttatggcagcactgcataattctcttactgtcatgccatccgtaagatgcttttctgtgactggtgagtactcaaccaagtcattctgagaatagtgtatgcggcgaccgagttgctcttgcccggcgtcaatacgggataataccgcgccacatagcagaactttaaaagtgctcatcattggaaaacgttcttcggggcgaaaactctcaaggatcttaccgctgttgagatccagttcgatgtaacccactcgtgcacccaactgatcttcagcatcttttactttcaccagcgtttctgggtgagcaaaaacaggaaggcaaaatgccgcaaaaaagggaataagggcgacacggaaatgttgaatactcatactcttcctttttcaatattattgaagcatttatcagggttattgtctcatgagcggatacatatttgaatgtatttagaaaaataaacaaataggggttccgcgcacatttccccgaaaagtgccacctgg

SEQ ID NO: 10 - DNA, 22 bp, synthetic construct
  source 1..22: mol_type = other DNA
gtcgagaattgagcttgcctcg

SEQ ID NO: 11 - DNA, 19 bp, synthetic construct
  source 1..19: mol_type = other DNA
ccaggtggcacttttcggg

SEQ ID NO: 12 - DNA, 51 bp, synthetic construct
  source 1..51: mol_type = other DNA
ccccgaaaagtgccacctgggatctaacatccaaagacgaaaggttgaatg

SEQ ID NO: 13 - DNA, 37 bp, synthetic construct
  source 1..37: mol_type = other DNA
cgtttcgaataattagttgttttttgatcttctcaag

SEQ ID NO: 14 - DNA, 49 bp, synthetic construct
  source 1..49: mol_type = other DNA
acaactaattattcgaaacgatgagattcccatctattttcactgctgt

SEQ ID NO: 15 - DNA, 50 bp, synthetic construct
  source 1..50: mol_type = other DNA
gcattctgacatcctcttgactaatgatgatgatgatgatgtgaactgcc

SEQ ID NO: 16 - DNA, 27 bp, synthetic construct
  source 1..27: mol_type = other DNA
tcaagaggatgtcagaatgccatttgc

SEQ ID NO: 17 - DNA, 42 bp, synthetic construct
  source 1..42: mol_type = other DNA
aggcaagctcaattctcgactacattcttcgcaggcttggct

SEQ ID NO: 18 - DNA, 5138 bp, synthetic construct
  source 1..5138: mol_type = other DNA
gtcgagaattgagcttgcctcgtccccgccgggtcacccggccagcgacatggaggcccagaataccctccttgacagtcttgacgtgcgcagctcaggggcatgatgtgactgtcgcccgtacatttagcccatacatccccatgtataatcatttgcatccatacattttgatggccgcacggcgcgaagcaaaaattacggctcctcgctgcagacctgcgagcagggaaacgctcccctcacagacgcgttgaattgtccccacgccgcgcccctgtagagaaatataaaaggttaggatttgccactgaggttcttctttcatatacttccttttaaaatcttgctaggatacagttctcacatcacatccgaacataaacaaaaatgggtaaggaaaagactcacgtttccagaccaagattgaactctaacatggacgctgacttgtacggttacaagtgggctagagacaacgttggtcaatctggtgctactatttacagattgtacggtaagccagacgctccagagttgttcttgaagcacggtaagggttctgttgctaacgacgttactgacgagatggttagattgaactggttgactgagttcatgccattgccaactattaagcacttcattagaactccagacgacgcttggttgttgactactgctattccaggtaagactgctttccaagttttggaggagtacccagactctggtgagaacattgttgacgctttggctgttttcttgagaagattgcactctattccagtttgtaactgtccattcaactctgacagagttttcagattggctcaagctcaatccagaatgaacaacggtttggttgacgcttctgacttcgacgacgagagaaacggttggccagttgagcaagtttggaaggagatgcacaagttgttgccattctctccagactctgttgttactcacggtgacttctctttggacaacttgattttcgacgagggtaagttgattggttgtattgacgttggtagagttggtattgctgacagataccaagacttggctattttgtggaactgtttgggtgagttctctccatctttgcaaaagagattgttccaaaagtacggtattgacaacccagacatgaacaagttgcaattccacttgatgttggacgagttcttctaaagtaactgacaataaaaagattcttgttttcaagaacttgtcatttgtatagtttttttatattgtagttgttctattttaatcaaatgttagcgtgatttatattttttttcgcctcgacatcatctgcccagatgcgaagttaagtgcgcagaaagtaatatcatgcgtcaatcgtatgtgaatgctggtcgctatactgctgtcgattcgatactaacgccgccatccagtgtcggatctgtgagcaaaaggccagcaaaaggccaggaaccgtaaaaaggccgcgttgctggcgtttttccataggctccgcccccctgacgagcatcacaaaaatcgacgctcaagtcagaggtgacgaaacccgacaggactataaagataccaggcgtttccccctggaagctccctcgtgcgctctcctgttccgaccctgccgcttaccggatacctgtccgcctttctcccttcgggaagcgtggcgctttctcatagctcacgctgtaggtatctcagttcggtgtaggtcgttcgctccaagctgggctgtgtgcacgaaccccccgttcagcccgaccgctgcgccttatccggtaactatcgtcttgagtccaacccggtaagacacgacttatcgccactggcagcagccactggtaacaggattagcagagcgaggtatgtaggcggtgctacagagttcttgaagtggtggcctaactacggctacactagaagaacagtatttggtatctgcgctctgctgaagccagttaccttcggaaaaagagttggtagctcttgatccggcaaacaaaccaccgctggtagcggtggtttttttgtttgcaagcagcagattacgcgcagaaaaaaaggatctcaagaagatcctttgatcttttctacggggtctgacgctcagtggaacgaaaactcacgttaagggattttggtcatgagattatcaaaaaggatcttcacctagatcctttttaattaaaaatgaagatttaaatcaatctaaagtatatatgagtaaacttggtctgacagttaccaatgcttaatcagtgaggcacctatctcagcgatctgtctatttcgttcatccatagttgcctgactccccgtcgtgtagataactacgatacgggagggcttaccatctggccccagtgctgcaatgataccgcgagatccacgctcaccggctccagatttatcagcaataaaccagccggccggaagggccgagcgcagaagtgggccggccactttatccgcctccatccagtctattaattgttgccgggaagctagagtaagtagttcgccagttaatagtttgcgcaacgttgttgccattgctacaggcatcgtggtgtcacgctcgtcgtttggtatggcttcattcagctccggttcccaacgatcaaggcgagttacatgatcccccatgttgtgcaaaaaagcggttagctccttcggtcctccgatcgttgtcagaagtaagttggccgcagtgttatcactcatggttatggcagcactgcataattctcttactgtcatgccatccgtaagatgcttttctgtgactggtgagtactcaaccaagtcattctgagaatagtgtatgcggcgaccgagttgctcttgcccggcgtcaatacgggataataccgcgccacatagcagaactttaaaagtgctcatcattggaaaacgttcttcggggcgaaaactctcaaggatcttaccgctgttgagatccagttcgatgtaacccactcgtgcacccaactgatcttcagcatcttttactttcaccagcgtttctgggtgagcaaaaacaggaaggcaaaatgccgcaaaaaagggaataagggcgacacggaaatgttgaatactcatactcttcctttttcaatattattgaagcatttatcagggttattgtctcatgagcggatacatatttgaatgtatttagaaaaataaacaaataggggttccgcgcacatttccccgaaaagtgccacctgggatctaacatccaaagacgaaaggttgaatgaaacctttttgccatccgacatccacaggtccattctcacacataagtgccaaacgcaacaggaggggatacactagcagcagaccgttgcaaacgcaggacctccactcctcttctcctcaacacccacttttgccatcgaaaaaccagcccagttattgggcttgattggagctcgctcattccaattccttctattaggctactaacaccatgactttattagcctgtctatcctggcccccctggcgaggttcatgtttgtttatttccgaatgcaacaagctccgcattacacccgaacatcactccagatgagggctttctgagtgtggggtcaaatagtttcatgttccccaaatggcccaaaactgacagtttaaacgctgtcttggaacctaatatgacaaaagcgtgatctcatccaagatgaactaagtttggttcgttgaaatgctaacggccagttggtcaaaaagaaacttccaaaagtcggcataccgtttgtcttgtttggtattgattgacgaatgctcaaaaataatctcattaatgcttagcgcagtctctctatcgcttctgaaccccggtgcacctgtgccgaaacgcaaatggggaaacacccgctttttggatgattatgcattgtctccacattgtatgcttccaagattctggtgggaatactgctgatagcctaacgttcatgatcaaaatttaactgttctaacccctacttgacagcaatatataaacagaaggaagctgccctgtcttaaacctttttttttatcatcattattagcttactttcataattgcgactggttccaattgacaagcttttgattttaacgacttttaacgacaacttgagaagatcaaaaaacaactaattattcgaaacgatgagattcccatctattttcactgctgttttgttcgctgcttcttctgctttggctgctccagttaacactactactgaggacgagactgctcaaattccagctgaggctgttattggttacttggacttggagggtgacttcgacgttgctgttttgccattctctaactctactaacaacggtttgttgttcattaacactactattgcttctattgctgctaaggaggagggtgtttctttggacaagagagaggctgaggctgttacattcccaggtgccctggttcctggcggagtcgctgatgctgctgcagcctataaagcagctaaagccggagccggtttaggtggtgtgccaggggtgggaggattaggtgtttcggcaggcgctgtcgttcctcaacccggagccggggtgaagcccggaaaagttcctggagtggggcttcctggagtttaccctggcggtgttttgcctggagccaggtttccgggtgttggtgttttgcccggagttccgactggcgccggtgtcaaacctaaagctccaggtgtgggtggtggcagttcacatcatcatcatcatcattagtcaagaggatgtcagaatgccatttgcctgagagatgcaggcttcatttttgatacttttttatttgtaacctatatagtataggattttttttgtcattttgtttcttctcgtacgagcttgctcctgatcagcctatctcgcagctgatgaatatcttgtggtaggggtttgggaaaatcattcgagtttgatgtttttcttggtatttcccactcctcttcagagtacagaagattaagtgacacgttcgtttgtgcaagcttcaacgatgccaaaagggtataataagcgtcatttgcagcattgtgaagaaaactatgtggcaagccaagcctgcgaagaatgta

SEQ ID NO: 19 - DNA, 24 bp, synthetic construct
  source 1..24: mol_type = other DNA
actgcagctttgatgcctgaaatc

SEQ ID NO: 20 - DNA, 20 bp, synthetic construct
  source 1..20: mol_type = other DNA
gggcgacagtcacatcatgc

SEQ ID NO: 21 - protein, 80 aa, synthetic construct
AAKAGAGLGGVPGVGGLGVSAGAVVPQPGAGVKPGKVPGVGLPGVYPGGVLPGARFPGVGVLPGVPTGAGVKPKAPGVGG

SEQ ID NO: 22 - DNA, 18 bp, synthetic construct
  source 1..18: mol_type = other DNA
gcagctaaagccggagcc

SEQ ID NO: 23 - DNA, 31 bp, synthetic construct
  source 1..31: mol_type = other DNA
ctaatgatgatgatgatgatgtgaactgcca

SEQ ID NO: 24 - DNA, 58 bp, synthetic construct
  source 1..58: mol_type = other DNA
ggcagttcacatcatcatcatcatcattagtcaagaggatgtcagaatgccatttgcc

SEQ ID NO: 25 - DNA, 50 bp, synthetic construct
  source 1..50: mol_type = other DNA
accacctaaaccggctccggctttagctgcagcctcagcctctctcttgt

SEQ ID NO: 26 - DNA, 5078 bp, synthetic construct
  source 1..5078: mol_type = other DNA
tcaagaggatgtcagaatgccatttgcctgagagatgcaggcttcatttttgatacttttttatttgtaacctatatagtataggattttttttgtcattttgtttcttctcgtacgagcttgctcctgatcagcctatctcgcagctgatgaatatcttgtggtaggggtttgggaaaatcattcgagtttgatgtttttcttggtatttcccactcctcttcagagtacagaagattaagtgacacgttcgtttgtgcaagcttcaacgatgccaaaagggtataataagcgtcatttgcagcattgtgaagaaaactatgtggcaagccaagcctgcgaagaatgtagtcgagaattgagcttgcctcgtccccgccgggtcacccggccagcgacatggaggcccagaataccctccttgacagtcttgacgtgcgcagctcaggggcatgatgtgactgtcgcccgtacatttagcccatacatccccatgtataatcatttgcatccatacattttgatggccgcacggcgcgaagcaaaaattacggctcctcgctgcagacctgcgagcagggaaacgctcccctcacagacgcgttgaattgtccccacgccgcgcccctgtagagaaatataaaaggttaggatttgccactgaggttcttctttcatatacttccttttaaaatcttgctaggatacagttctcacatcacatccgaacataaacaaaaatgggtaaggaaaagactcacgtttccagaccaagattgaactctaacatggacgctgacttgtacggttacaagtgggctagagacaacgttggtcaatctggtgctactatttacagattgtacggtaagccagacgctccagagttgttcttgaagcacggtaagggttctgttgctaacgacgttactgacgagatggttagattgaactggttgactgagttcatgccattgccaactattaagcacttcattagaactccagacgacgcttggttgttgactactgctattccaggtaagactgctttccaagttttggaggagtacccagactctggtgagaacattgttgacgctttggctgttttcttgagaagattgcactctattccagtttgtaactgtccattcaactctgacagagttttcagattggctcaagctcaatccagaatgaacaacggtttggttgacgcttctgacttcgacgacgagagaaacggttggccagttgagcaagtttggaaggagatgcacaagttgttgccattctctccagactctgttgttactcacggtgacttctctttggacaacttgattttcgacgagggtaagttgattggttgtattgacgttggtagagttggtattgctgacagataccaagacttggctattttgtggaactgtttgggtgagttctctccatctttgcaaaagagattgttccaaaagtacggtattgacaacccagacatgaacaagttgcaattccacttgatgttggacgagttcttctaaagtaactgacaataaaaagattcttgttttcaagaacttgtcatttgtatagtttttttatattgtagttgttctattttaatcaaatgttagcgtgatttatattttttttcgcctcgacatcatctgcccagatgcgaagttaagtgcgcagaaagtaatatcatgcgtcaatcgtatgtgaatgctggtcgctatactgctgtcgattcgatactaacgccgccatccagtgtcggatctgtgagcaaaaggccagcaaaaggccaggaaccgtaaaaaggccgcgttgctggcgtttttccataggctccgcccccctgacgagcatcacaaaaatcgacgctcaagtcagaggtgacgaaacccgacaggactataaagataccaggcgtttccccctggaagctccctcgtgcgctctcctgttccgaccctgccgcttaccggatacctgtccgcctttctcccttcgggaagcgtggcgctttctcatagctcacgctgtaggtatctcagttcggtgtaggtcgttcgctccaagctgggctgtgtgcacgaaccccccgttcagcccgaccgctgcgccttatccggtaactatcgtcttgagtccaacccggtaagacacgacttatcgccactggcagcagccactggtaacaggattagcagagcgaggtatgtaggcggtgctacagagttcttgaagtggtggcctaactacggctacactagaagaacagtatttggtatctgcgctctgctgaagccagttaccttcggaaaaagagttggtagctcttgatccggcaaacaaaccaccgctggtagcggtggtttttttgtttgcaagcagcagattacgcgcagaaaaaaaggatctcaagaagatcctttgatcttttctacggggtctgacgctcagtggaacgaaaactcacgttaagggattttggtcatgagattatcaaaaaggatcttcacctagatcctttttaattaaaaatgaagatttaaatcaatctaaagtatatatgagtaaacttggtctgacagttaccaatgcttaatcagtgaggcacctatctcagcgatctgtctatttcgttcatccatagttgcctgactccccgtcgtgtagataactacgatacgggagggcttaccatctggccccagtgctgcaatgataccgcgagatccacgctcaccggctccagatttatcagcaataaaccagccggccggaagggccgagcgcagaagtgggccggccactttatccgcctccatccagtctattaattgttgccgggaagctagagtaagtagttcgccagttaatagtttgcgcaacgttgttgccattgctacaggcatcgtggtgtcacgctcgtcgtttggtatggcttcattcagctccggttcccaacgatcaaggcgagttacatgatcccccatgttgtgcaaaaaagcggttagctccttcggtcctccgatcgttgtcagaagtaagttggccgcagtgttatcactcatggttatggcagcactgcataattctcttactgtcatgccatccgtaagatgcttttctgtgactggtgagtactcaaccaagtcattctgagaatagtgtatgcggcgaccgagttgctcttgcccggcgtcaatacgggataataccgcgccacatagcagaactttaaaagtgctcatcattggaaaacgttcttcggggcgaaaactctcaaggatcttaccgctgttgagatccagttcgatgtaacccactcgtgcacccaactgatcttcagcatcttttactttcaccagcgtttctgggtgagcaaaaacaggaaggcaaaatgccgcaaaaaagggaataagggcgacacggaaatgttgaatactcatactcttcctttttcaatattattgaagcatttatcagggttattgtctcatgagcggatacatatttgaatgtatttagaaaaataaacaaataggggttccgcgcacatttccccgaaaagtgccacctgggatctaacatccaaagacgaaaggttgaatgaaacctttttgccatccgacatccacaggtccattctcacacataagtgccaaacgcaacaggaggggatacactagcagcagaccgttgcaaacgcaggacctccactcctcttctcctcaacacccacttttgccatcgaaaaaccagcccagttattgggcttgattggagctcgctcattccaattccttctattaggctactaacaccatgactttattagcctgtctatcctggcccccctggcgaggttcatgtttgtttatttccgaatgcaacaagctccgcattacacccgaacatcactccagatgagggctttctgagtgtggggtcaaatagtttcatgttccccaaatggcccaaaactgacagtttaaacgctgtcttggaacctaatatgacaaaagcgtgatctcatccaagatgaactaagtttggttcgttgaaatgctaacggccagttggtcaaaaagaaacttccaaaagtcggcataccgtttgtcttgtttggtattgattgacgaatgctcaaaaataatctcattaatgcttagcgcagtctctctatcgcttctgaaccccggtgcacctgtgccgaaacgcaaatggggaaacacccgctttttggatgattatgcattgtctccacattgtatgcttccaagattctggtgggaatactgctgatagcctaacgttcatgatcaaaatttaactgttctaacccctacttgacagcaatatataaacagaaggaagctgccctgtcttaaacctttttttttatcatcattattagcttactttcataattgcgactggttccaattgacaagcttttgattttaacgacttttaacgacaacttgagaagatcaaaaaacaactaattattcgaaacgatgagattcccatctattttcactgctgttttgttcgctgcttcttctgctttggctgctccagttaacactactactgaggacgagactgctcaaattccagctgaggctgttattggttacttggacttggagggtgacttcgacgttgctgttttgccattctctaactctactaacaacggtttgttgttcattaacactactattgcttctattgctgctaaggaggagggtgtttctttggacaagagagaggctgaggctgcagctaaagccggagccggtttaggtggtgtgccaggggtgggaggattaggtgtttcggcaggcgctgtcgttcctcaacccggagccggggtgaagcccggaaaagttcctggagtggggcttcctggagtttaccctggcggtgttttgcctggagccaggtttccgggtgttggtgttttgcccggagttccgactggcgccggtgtcaaacctaaagctccaggtgtgggtggtggcagttcacatcatcatcatcatcattag

SEQ ID NO: 27 - DNA, 23 bp, synthetic construct
  source 1..23: mol_type = other DNA
agctttgatgcctgaaatcccag

SEQ ID NO: 28 - DNA, 23 bp, synthetic construct
  source 1..23: mol_type = other DNA
gcctgccgaaacacctaatcctc

SEQ ID NO: 29 - protein, 89 aa, synthetic construct
AAKAGAGLGGVPGVGGLGVSAGAVVPQPGAGVKPGKVPGVGLPGVYPGGVLPGARFPGVGVLPGVPTGAGVKPKAPGVGGGSSHHHHHH

SEQ ID NO: 30 - protein, 9 aa, synthetic construct
GSSHHHHHH

SEQ ID NO: 31 - DNA, 270 bp, synthetic construct
  source 1..270: mol_type = other DNA
gcagctaaagccggagccggtttaggtggtgtgccaggggtgggaggattaggtgtttcggcaggcgctgtcgttcctcaacccggagccggggtgaagcccggaaaagttcctggagtggggcttcctggagtttaccctggcggtgttttgcctggagccaggtttccgggtgttggtgttttgcccggagttccgactggcgccggtgtcaaacctaaagctccaggtgtgggtggtggcagttcacatcatcatcatcatcattag

SEQ ID NO: 32 - DNA, 22 bp, synthetic construct
  source 1..22: mol_type = other DNA
ggttgtgtcaccagaagcagct

SEQ ID NO: 33 - DNA, 23 bp, synthetic construct
  source 1..23: mol_type = other DNA
ccgtaagtaggaatgcctccaac

SEQ ID NO: 34 - DNA, 22 bp, synthetic construct
  source 1..22: mol_type = other DNA
gttggagagaaaggtgacgagg

SEQ ID NO: 35 - DNA, 22 bp, synthetic construct
  source 1..22: mol_type = other DNA
tggtctcccttttcacccacag

SEQ ID NO: 36 - DNA, 22 bp, synthetic construct
  source 1..22: mol_type = other DNA
tgttgacggcttacctggagac

SEQ ID NO: 37 - DNA, 22 bp, synthetic construct
  source 1..22: mol_type = other DNA
ggtagaccaactccaggctctc

SEQ ID NO: 38 - DNA, 22 bp, synthetic construct
  source 1..22: mol_type = other DNA
gattccctggacctaaaggtgc

SEQ ID NO: 39 - DNA, 22 bp, synthetic construct
  source 1..22: mol_type = other DNA
agcctctccatctttgccagca

SEQ ID NO: 40 - DNA, 21 bp, synthetic construct
  source 1..21: mol_type = other DNA
tgatccccaatgcttcacaag

SEQ ID NO: 41 - DNA, 23 bp, synthetic construct
  source 1..23: mol_type = other DNA
gccaagtaacggtagtaatctcc